European Patent Specification EP 3 807 293 B1, published January 14, 2026. Title: Peptides Having Antiperspirant Activity. Applicant: AZIENDE CHIMICHE RIUNITE ANGELINI FRANCESCO - A.C.R.A.F. S.P.A. The sequence listing filed with the application follows.

SEQUENCE LISTING (5 sequences)

SEQ ID NO: 1 - protein, 9 aa, Artificial Sequence
  None
HYWRELQYR

SEQ ID NO: 2 - protein, 14 aa, Artificial Sequence
  None
MQVWLRMWIDYRAT

SEQ ID NO: 3 - protein, 10 aa, Artificial Sequence
  None
RRVVLVNNIL

SEQ ID NO: 4 - protein, 10 aa, Artificial Sequence
  None
LRVQMVNMFL

SEQ ID NO: 5 - protein, 8 aa, Artificial Sequence
  None
WEQEFLRR